European Patent Specification EP 3 921 419 B1, published April 8, 2026. Title: SIRT2-ABLATED CHIMERIC T CELLS. Applicant: H. Lee Moffitt Cancer Center and Research Institute, Inc. The sequence listing filed with the application follows.

SEQUENCE LISTING (14 sequences)

SEQ ID NO: 1 - protein, 15 aa, Artificial Sequence
  Synthetic Construct
GILAADESTGSIAKR

SEQ ID NO: 2 - protein, 23 aa, Artificial Sequence
  Synthetic Construct
SCNCLLLKVNQIGSVTESLQACK

SEQ ID NO: 3 - protein, 14 aa, Artificial Sequence
  Synthetic Construct
FIIPNIVKYSPHCK

SEQ ID NO: 4 - protein, 30 aa, Artificial Sequence
  Synthetic Construct
SVVLMSHLGRPDGVPMPDKYSLEPVAAELK

SEQ ID NO: 5 - protein, 27 aa, Artificial Sequence
  Synthetic Construct
WGEAGAEYVVESTGVFTTMEKAGAHLK

SEQ ID NO: 6 - protein, 14 aa, Artificial Sequence
  Synthetic Construct
CCSGAIIVLTKSGR

SEQ ID NO: 7 - protein, 46 aa, Artificial Sequence
  Synthetic Construct
NFTGRNDANPETHAFVTSPEIVTALAIAGTLKFNPETDFLTGKDGK

SEQ ID NO: 8 - protein, 19 aa, Artificial Sequence
  Synthetic Construct
NILGGTVFREPIICKNIPR

SEQ ID NO: 9 - protein, 11 aa, Artificial Sequence
  Synthetic Construct
SSDEAYAIAKK

SEQ ID NO: 10 - protein, 12 aa, Artificial Sequence
  Synthetic Construct
ISQLYGDLKHLK

SEQ ID NO: 11 - protein, 16 aa, Artificial Sequence
  Synthetic Construct
ETECTYFSTPLLLGKK

SEQ ID NO: 12 - protein, 12 aa, Artificial Sequence
  Synthetic Construct
GQQQVFKGLNDK

SEQ ID NO: 13 - protein, 9 aa, Artificial Sequence
  Synthetic Construct
FITALKSTG

SEQ ID NO: 14 - protein, 7 aa, Artificial Sequence
  Synthetic Construct
LTFKYER